European Patent Application EP 4 219 715 A2, published August 2, 2023. Title: STABILIZED CEBPA SARNA COMPOSITIONS AND METHODS OF USE. Applicant: MINA THERAPEUTICS LIMITED. Application EP. The sequence listing filed with the application follows.

SEQUENCE LISTING (23 sequences)

SEQ ID NO: 1 - DNA, 4001 bp, Homo sapiens
  source 1..4001: mol_type = genomic DNA
tccctctcccaccaggggtatacatcctcagagctgacccacgacctagctttctggtgtgactcggggtgggggctcccactggtcacctggtgacccccatcgcagtgagttccgccccaaggggaagcccagcctatagcaggctggggtggggtgtgtgcggagggaggtgggagaggcgtggaactagagaccctccaccttcatgtagaactaggggaacaaccttaggttccaagccccaagtccctatgtttccacccctttctaaggacaggcgtggaggagcggctggggctggcgggcttgtcgggatctcagctccctgagccctcctcctgccacgggcctgctcccctccttctctcatgggggtctgctgtagcctcgggaaggaggcaggaaacctccaaataaaatgacaaggcacgatttgctccccctactcagtaggcattggagcggtgagtttgcatttccaaggcacaaggttatcctaaatactagagttgccgggctcccagctcagccccaagaattctcccctcctcgcagggagaagccaccgcctggccccctcatcttagacgcaccaagtccggcgcagaggaagggaggggacacgcggagcaggccaggctttcaggaggcaccggaatctcctagtcctggctcgcacggctcgggcaagcctcgagatccggcgaccccaaaccactccctgggtccccgccggaggctggcccagggcggtcccacagccgcgcgcctcacgcgcagttgcccatggccttgaccaaggagctctctggcagctggcggaagatgccccgcagcgtgtccagttcgcggctcagctgttccacccgcttgcgcaggcggtcattgtcactggtcagctccagcaccttctgctgcgtctccacgttgcgctgcttggccttgtcgcggctcttgcgcaccgcgatgttgttgcgctcgcgccgcacccggtactcgttgctgttcttgtccaccgacttcttggccttgcccgcgccgctgccgccactcgcgcggaggtcggggtgcgcggcgcccagccccttgagcgcgctgccagggcccggcaggccggcggcaccgagcgcgggcgcggggtgcgggctgggcacgggcgtgggcggcggcgtggggtgaccgggctgcaggtgcatggtggtctggccgcagtgcgcgatctggaactgcaggtgcggggcggccaggtgcgcgggcggcgggtgcgggtgcgggtgcgagggcggcggcggcggcggcggctggtaagggaagaggccggccagcgccagctgcttggcttcatcctcctcgcggggctcctgcttgatcaccagcggccgcagcgccggcgccccgacgcgctcgtacaggggctccagcctgccgtccaggtagccggcggccgcgcagccgtagccgggcgggggcccgtgcgctcccccgggcatgacggcgccgccggggcccgcgggcgcgcccgggtagtcaaagtcgccgccgccgccgccgcccgtggggcccacggccgccttggccttctcctgctgccggctgtgctggaacaggtcggccaggaactcgtcgttgaaggcggccgggtcgatgtaggcgctgatgtcgatggacgtctcgtgctcgcagatgccgcccagcggctccggggcggcaggtggggcgggaggctgcgcggggcccgcgccccggggaaagccgaaggcggcgctgctgggcgcgtgcggggggctctgcaggtggctgctcatcgggggccgcggctccgcctcgtagaagtcggccgactccatgggggagttagagttctcccggcatggcgagcctcggcggcctccagcctgcgcggggcgtcgccgccgcccacccggagaccctgctcgcccgcgcccgcgcacctccgggtcgcgaatggcccggcccgcgccggcccagcttttatacccggcaggccgcgtcgccccctagagtccgaggcggcctctgtccccgggctgcggcggcgcggcgcctgctgggtcctagcgcgcggccggcatggggcggcgaaccagcgcggcacagcgccgcgctccccaggcaggccgcggcgcaacgcccaccgcctccagcgcgcccagcagagccgcggcgctcgctccaagctccgcccccggcccggccgtcgcccccgcgcccacgtggtcggtagcgggggccccctcctcctgcctgccctaggcgcccgtatccagccacggccgggagcccaggagtatcccgaggctgcacggggtaggggtggggggcggagggcgagtcttggtcttgagctgctggggcgcggattctctttcaaagccagaaccaggcctgtcccggacccgcgtcccggggaggctgcagcgcagagcagcggggctggggccggtggggggccgtttgggacgcgcggagaggtcctgagcgcggtggctctgcgtctcctagctctgatctccaggctacccctgtgattccgcgcagaggtacctctcggaggacgccggggtcccatgggcggcgccgcgcagggcgctaggaccccgcggggagcggaggcggcctcggcccgggagcctggaggacctggccggtcgatccgcccgggctggaaaactttctttataattacttctccaggtcggagcgcgcggcttgctaggcgcgcggggccggcgctgttacccggcgtggagtcgccgattttttttcctgcgggaccgcggggccccccagactagcggagctggacgccggggcgagcacggggaggggcgcaccgagggaggagacaaacttaactctggggccgggattccgaggcgggggccgcagccctcgaggcccgaagccaccgcttcctcccccgcctccccattcaggtgggcgccaacggcgggagcgagggtgtccaggccgccgggctgccaggtccgagcacgcacagggagaactctgcccagtggttcgccgggcgctgtagtccccgggatcctagggaccgaggcggccaggccctggggccccttgagtgcggcagctaatgctctcaccgcggcgggggaaggagcttgccaccgagacccccagccacgtgcgtccctcgcattctttaccggggccggggtggcggctacggaccgtcagctgggcccagatggagtcttgggagccctcaagtgtctcctgtccttgcccgcgccgcccctcgccactggcgctgaggcctgacgccgcctgcgtcccggctagaggcgcgcttgcctacaggtgagggaagacccccttcaccgacagtggccttaggcctggcaaggcgccacgacccgcccaggagccccggagggggcacagctaaaaacaccgctggagagccccgagcttccacgacgatcgcagtaaagaagcagtttcatctgggcaacgcacactgcgctttaatcaagttcctattcaacatagtcccagtgattaatagcccaactgcttcgttttcggtccagagctcataaacaagatatttttagcttgacgcttttggacgggagggagtaaaaaccagatacgttaaataaatatcccgatgtgagccggagagctgcttgctgagccaaatgcaggacccattcatatagcattcacctgtggagggagacctggacggaaatcaaaaagcaccaagagcgatttgcgtttttttctgcggtgctaaaactaatggcttttcctacctaggaacaaagaaacgccactgtacatgcacggttcccggcctgtggagttgtgggaggaaggcgatgtctggccttttttgcacagctgctgttgcctgcccagagatcgggaactctgccccgtaggactggaagaaacctcagtaatgggaataagactttgtccaatagggggctgatgaatgtgtg

SEQ ID NO: 2 - RNA, 21 nt, synthetic construct
  source 1..21: mol_type = other RNA
gcggtcattgtcactggtctt

SEQ ID NO: 3 - RNA, 21 nt, synthetic construct
  source 1..21: mol_type = other RNA
gaccagtgacaatgaccgctt

SEQ ID NO: 4 - DNA, 22 bp, synthetic construct
  misc_feature 22: note = DNA
  misc_feature >1: note = 5' NH2-(C6H12)-linker
  misc_feature 22: note = Inverted nucleotide
  source 1..22: mol_type = other DNA
  misc_feature 1..21: note = RNA
gcggtcattgtcactggtcttt

SEQ ID NO: 5 - RNA, 21 nt, synthetic construct
  misc_feature 20^21: note = Phosphorothioate linkage
  source 1..21: mol_type = other RNA
gaccagtgacaatgaccgctt

SEQ ID NO: 6 - DNA, 22 bp, synthetic construct
  misc_feature 22: note = DNA
  misc_feature >1: note = 5' NH2-(C6H12)-linker
  modified_base 1: mod_base = OTHER; note = 2'-Fluoro nucleotide
  modified_base 2: mod_base = OTHER; note = 2'-O-Methyl nucleotide
  modified_base 3: mod_base = OTHER; note = 2'-Fluoro nucleotide
  modified_base 4: mod_base = OTHER; note = 2'-O-Methyl nucleotide
  modified_base 5: mod_base = OTHER; note = 2'-Fluoro nucleotide
  modified_base 6: mod_base = OTHER; note = 2'-O-Methyl nucleotide
  modified_base 7: mod_base = OTHER; note = 2'-Fluoro nucleotide
  modified_base 8: mod_base = OTHER; note = 2'-O-Methyl nucleotide
  modified_base 9: mod_base = OTHER; note = 2'-Fluoro nucleotide
  modified_base 10: mod_base = OTHER; note = 2'-O-Methyl nucleotide
  modified_base 11: mod_base = OTHER; note = 2'-Fluoro nucleotide
  modified_base 12: mod_base = OTHER; note = 2'-O-Methyl nucleotide
  modified_base 13: mod_base = OTHER; note = 2'-Fluoro nucleotide
  modified_base 14: mod_base = OTHER; note = 2'-O-Methyl nucleotide
  modified_base 15: mod_base = OTHER; note = 2'-Fluoro nucleotide
  modified_base 16: mod_base = OTHER; note = 2'-O-Methyl nucleotide
  modified_base 17: mod_base = OTHER; note = 2'-Fluoro nucleotide
  modified_base 18: mod_base = OTHER; note = 2'-O-Methyl nucleotide
  modified_base 19: mod_base = OTHER; note = 2'-Fluoro nucleotide
  modified_base 20..21: mod_base = OTHER; note = 2'-O-Methyl nucleotide
  misc_feature 22: note = Inverted nucleotide
  source 1..22: mol_type = other DNA
  misc_feature 1..21: note = RNA
gcggtcattgtcactggtcttt

SEQ ID NO: 7 - RNA, 21 nt, synthetic construct
  modified_base 1: mod_base = OTHER; note = 2'-O-Methyl nucleotide
  modified_base 2: mod_base = OTHER; note = 2'-Fluoro nucleotide
  modified_base 3: mod_base = OTHER; note = 2'-O-Methyl nucleotide
  modified_base 4: mod_base = OTHER; note = 2'-Fluoro nucleotide
  modified_base 5: mod_base = OTHER; note = 2'-O-Methyl nucleotide
  modified_base 6: mod_base = OTHER; note = 2'-Fluoro nucleotide
  modified_base 7: mod_base = OTHER; note = 2'-O-Methyl nucleotide
  modified_base 8: mod_base = OTHER; note = 2'-Fluoro nucleotide
  modified_base 9: mod_base = OTHER; note = 2'-O-Methyl nucleotide
  modified_base 10: mod_base = OTHER; note = 2'-Fluoro nucleotide
  modified_base 11: mod_base = OTHER; note = 2'-O-Methyl nucleotide
  modified_base 12: mod_base = OTHER; note = 2'-Fluoro nucleotide
  modified_base 13: mod_base = OTHER; note = 2'-O-Methyl nucleotide
  modified_base 14: mod_base = OTHER; note = 2'-Fluoro nucleotide
  modified_base 15: mod_base = OTHER; note = 2'-O-Methyl nucleotide
  modified_base 16: mod_base = OTHER; note = 2'-Fluoro nucleotide
  modified_base 17: mod_base = OTHER; note = 2'-O-Methyl nucleotide
  modified_base 18: mod_base = OTHER; note = 2'-Fluoro nucleotide
  modified_base 19..21: mod_base = OTHER; note = 2'-O-Methyl nucleotide
  misc_feature 20^21: note = Phosphorothioate linkage
  source 1..21: mol_type = other RNA
gaccagtgacaatgaccgctt

SEQ ID NO: 8 - DNA, 22 bp, synthetic construct
  misc_feature 22: note = DNA
  misc_feature >1: note = 5' NH2-(C6H12)-linker
  modified_base 1: mod_base = OTHER; note = 2'-Fluoro nucleotide
  modified_base 2: mod_base = OTHER; note = 2'-O-Methyl nucleotide
  modified_base 3: mod_base = OTHER; note = 2'-Fluoro nucleotide
  modified_base 4: mod_base = OTHER; note = 2'-O-Methyl nucleotide
  modified_base 5: mod_base = OTHER; note = 2'-Fluoro nucleotide
  modified_base 6: mod_base = OTHER; note = 2'-O-Methyl nucleotide
  modified_base 7: mod_base = OTHER; note = 2'-Fluoro nucleotide
  modified_base 8: mod_base = OTHER; note = 2'-O-Methyl nucleotide
  modified_base 9: mod_base = OTHER; note = 2'-Fluoro nucleotide
  modified_base 10: mod_base = OTHER; note = 2'-O-Methyl nucleotide
  modified_base 11: mod_base = OTHER; note = 2'-Fluoro nucleotide
  modified_base 12: mod_base = OTHER; note = 2'-O-Methyl nucleotide
  modified_base 13: mod_base = OTHER; note = 2'-Fluoro nucleotide
  modified_base 14: mod_base = OTHER; note = 2'-O-Methyl nucleotide
  modified_base 15: mod_base = OTHER; note = 2'-Fluoro nucleotide
  modified_base 16: mod_base = OTHER; note = 2'-O-Methyl nucleotide
  modified_base 17: mod_base = OTHER; note = 2'-Fluoro nucleotide
  modified_base 18: mod_base = OTHER; note = 2'-O-Methyl nucleotide
  modified_base 19: mod_base = OTHER; note = 2'-Fluoro nucleotide
  modified_base 20..21: mod_base = OTHER; note = 2'-O-Methyl nucleotide
  misc_feature 22: note = Inverted nucleotide
  source 1..22: mol_type = other DNA
  misc_feature 1..21: note = RNA
gcggtcattgtcactggtcttt

SEQ ID NO: 9 - RNA, 21 nt, synthetic construct
  modified_base 1: mod_base = OTHER; note = 2'-O-Methyl nucleotide
  modified_base 2: mod_base = OTHER; note = 2'-Fluoro nucleotide
  modified_base 3: mod_base = OTHER; note = 2'-O-Methyl nucleotide
  modified_base 4: mod_base = OTHER; note = 2'-Fluoro nucleotide
  modified_base 5: mod_base = OTHER; note = 2'-O-Methyl nucleotide
  modified_base 6: mod_base = OTHER; note = 2'-Fluoro nucleotide
  modified_base 7: mod_base = OTHER; note = 2'-O-Methyl nucleotide
  modified_base 8: mod_base = OTHER; note = 2'-Fluoro nucleotide
  modified_base 9: mod_base = OTHER; note = 2'-O-Methyl nucleotide
  modified_base 10: mod_base = OTHER; note = 2'-Fluoro nucleotide
  modified_base 11: mod_base = OTHER; note = 2'-O-Methyl nucleotide
  modified_base 12: mod_base = OTHER; note = 2'-Fluoro nucleotide
  modified_base 13: mod_base = OTHER; note = 2'-O-Methyl nucleotide
  modified_base 14: mod_base = OTHER; note = 2'-Fluoro nucleotide
  modified_base 15: mod_base = OTHER; note = 2'-O-Methyl nucleotide
  modified_base 16: mod_base = OTHER; note = 2'-Fluoro nucleotide
  modified_base 17: mod_base = OTHER; note = 2'-O-Methyl nucleotide
  modified_base 18: mod_base = OTHER; note = 2'-Fluoro nucleotide
  modified_base 19..21: mod_base = OTHER; note = 2'-O-Methyl nucleotide
  misc_feature 19..21: note = Phosphorothioate linkage
  source 1..21: mol_type = other RNA
gaccagtgacaatgaccgctt

SEQ ID NO: 10 - DNA, 22 bp, synthetic construct
  misc_feature 22: note = DNA
  misc_feature >1: note = 5' NH2-(C6H12)-linker
  modified_base 1: mod_base = OTHER; note = 2'-Fluoro nucleotide
  modified_base 2: mod_base = OTHER; note = 2'-O-Methyl nucleotide
  modified_base 3: mod_base = OTHER; note = 2'-Fluoro nucleotide
  modified_base 4: mod_base = OTHER; note = 2'-O-Methyl nucleotide
  modified_base 5: mod_base = OTHER; note = 2'-Fluoro nucleotide
  modified_base 6: mod_base = OTHER; note = 2'-O-Methyl nucleotide
  modified_base 7: mod_base = OTHER; note = 2'-Fluoro nucleotide
  modified_base 8: mod_base = OTHER; note = 2'-O-Methyl nucleotide
  modified_base 9..11: mod_base = OTHER; note = 2'-Fluoro nucleotide
  modified_base 12: mod_base = OTHER; note = 2'-O-Methyl nucleotide
  modified_base 13: mod_base = OTHER; note = 2'-Fluoro nucleotide
  modified_base 14: mod_base = OTHER; note = 2'-O-Methyl nucleotide
  modified_base 15: mod_base = OTHER; note = 2'-Fluoro nucleotide
  modified_base 16: mod_base = OTHER; note = 2'-O-Methyl nucleotide
  modified_base 17: mod_base = OTHER; note = 2'-Fluoro nucleotide
  modified_base 18: mod_base = OTHER; note = 2'-O-Methyl nucleotide
  modified_base 19: mod_base = OTHER; note = 2'-Fluoro nucleotide
  modified_base 20..21: mod_base = OTHER; note = 2'-O-Methyl nucleotide
  misc_feature 22: note = Inverted nucleotide
  source 1..22: mol_type = other DNA
  misc_feature 1..21: note = RNA
gcggtcattgtcactggtcttt

SEQ ID NO: 11 - RNA, 21 nt, synthetic construct
  modified_base 1: mod_base = OTHER; note = 2'-O-Methyl nucleotide
  modified_base 2: mod_base = OTHER; note = 2'-Fluoro nucleotide
  modified_base 3: mod_base = OTHER; note = 2'-O-Methyl nucleotide
  modified_base 4: mod_base = OTHER; note = 2'-Fluoro nucleotide
  modified_base 5: mod_base = OTHER; note = 2'-O-Methyl nucleotide
  modified_base 6: mod_base = OTHER; note = 2'-Fluoro nucleotide
  modified_base 7: mod_base = OTHER; note = 2'-O-Methyl nucleotide
  modified_base 8: mod_base = OTHER; note = 2'-Fluoro nucleotide
  modified_base 9..11: mod_base = OTHER; note = 2'-O-Methyl nucleotide
  modified_base 12: mod_base = OTHER; note = 2'-Fluoro nucleotide
  modified_base 13: mod_base = OTHER; note = 2'-O-Methyl nucleotide
  modified_base 14: mod_base = OTHER; note = 2'-Fluoro nucleotide
  modified_base 15: mod_base = OTHER; note = 2'-O-Methyl nucleotide
  modified_base 16: mod_base = OTHER; note = 2'-Fluoro nucleotide
  modified_base 17: mod_base = OTHER; note = 2'-O-Methyl nucleotide
  modified_base 18: mod_base = OTHER; note = 2'-Fluoro nucleotide
  modified_base 19..21: mod_base = OTHER; note = 2'-O-Methyl nucleotide
  misc_feature 19..21: note = Phosphorothioate linkage
  source 1..21: mol_type = other RNA
gaccagtgacaatgaccgctt

SEQ ID NO: 12 - DNA, 22 bp, synthetic construct
  misc_feature 1..21: note = RNA
  misc_feature 22: note = DNA
  misc_feature >1: note = 5' NH2-(C6H12)-linker
  modified_base 1: mod_base = OTHER; note = 2'-Fluoro nucleotide
  modified_base 2: mod_base = OTHER; note = 2'-O-Methyl nucleotide
  modified_base 3: mod_base = OTHER; note = 2'-Fluoro nucleotide
  modified_base 4: mod_base = OTHER; note = 2'-O-Methyl nucleotide
  modified_base 5: mod_base = OTHER; note = 2'-Fluoro nucleotide
  modified_base 6: mod_base = OTHER; note = 2'-O-Methyl nucleotide
  modified_base 7: mod_base = OTHER; note = 2'-Fluoro nucleotide
  modified_base 8: mod_base = OTHER; note = 2'-O-Methyl nucleotide
  modified_base 9..11: mod_base = OTHER; note = 2'-Fluoro nucleotide
  modified_base 12: mod_base = OTHER; note = 2'-O-Methyl nucleotide
  modified_base 13: mod_base = OTHER; note = 2'-Fluoro nucleotide
  modified_base 14: mod_base = OTHER; note = 2'-O-Methyl nucleotide
  modified_base 15: mod_base = OTHER; note = 2'-Fluoro nucleotide
  modified_base 16: mod_base = OTHER; note = 2'-O-Methyl nucleotide
  modified_base 17: mod_base = OTHER; note = 2'-Fluoro nucleotide
  modified_base 18: mod_base = OTHER; note = 2'-O-Methyl nucleotide
  modified_base 19: mod_base = OTHER; note = 2'-Fluoro nucleotide
  modified_base 20..21: mod_base = OTHER; note = 2'-O-Methyl nucleotide
  misc_feature 22: note = Inverted nucleotide
  source 1..22: mol_type = other DNA
gcggtcatacacactggtcttt

SEQ ID NO: 13 - RNA, 21 nt, synthetic construct
  modified_base 1: mod_base = OTHER; note = 2'-O-Methyl nucleotide
  modified_base 2: mod_base = OTHER; note = 2'-Fluoro nucleotide
  modified_base 3: mod_base = OTHER; note = 2'-O-Methyl nucleotide
  modified_base 4: mod_base = OTHER; note = 2'-Fluoro nucleotide
  modified_base 5: mod_base = OTHER; note = 2'-O-Methyl nucleotide
  modified_base 6: mod_base = OTHER; note = 2'-Fluoro nucleotide
  modified_base 7: mod_base = OTHER; note = 2'-O-Methyl nucleotide
  modified_base 8: mod_base = OTHER; note = 2'-Fluoro nucleotide
  modified_base 9..11: mod_base = OTHER; note = 2'-O-Methyl nucleotide
  modified_base 12: mod_base = OTHER; note = 2'-Fluoro nucleotide
  modified_base 13: mod_base = OTHER; note = 2'-O-Methyl nucleotide
  modified_base 14: mod_base = OTHER; note = 2'-Fluoro nucleotide
  modified_base 15: mod_base = OTHER; note = 2'-O-Methyl nucleotide
  modified_base 16: mod_base = OTHER; note = 2'-Fluoro nucleotide
  modified_base 17: mod_base = OTHER; note = 2'-O-Methyl nucleotide
  modified_base 18: mod_base = OTHER; note = 2'-Fluoro nucleotide
  modified_base 19..21: mod_base = OTHER; note = 2'-O-Methyl nucleotide
  misc_feature 19..21: note = Phosphorothioate linkage
  source 1..21: mol_type = other RNA
gaccagtgtgtatgaccgctt

SEQ ID NO: 14 - DNA, 22 bp, synthetic construct
  misc_feature 1..21: note = RNA
  misc_feature 22: note = DNA
  misc_feature >1: note = 5' NH2-(C6H12)-linker
  modified_base 1: mod_base = OTHER; note = 2'-Fluoro nucleotide
  modified_base 2: mod_base = OTHER; note = 2'-O-Methyl nucleotide
  modified_base 3: mod_base = OTHER; note = 2'-Fluoro nucleotide
  modified_base 4: mod_base = OTHER; note = 2'-O-Methyl nucleotide
  modified_base 5: mod_base = OTHER; note = 2'-Fluoro nucleotide
  modified_base 6: mod_base = OTHER; note = 2'-O-Methyl nucleotide
  modified_base 7..9: mod_base = OTHER; note = 2'-Fluoro nucleotide
  modified_base 10: mod_base = OTHER; note = 2'-O-Methyl nucleotide
  modified_base 11: mod_base = OTHER; note = 2'-Fluoro nucleotide
  modified_base 12: mod_base = OTHER; note = 2'-O-Methyl nucleotide
  modified_base 13: mod_base = OTHER; note = 2'-Fluoro nucleotide
  modified_base 14: mod_base = OTHER; note = 2'-O-Methyl nucleotide
  modified_base 15: mod_base = OTHER; note = 2'-Fluoro nucleotide
  modified_base 16: mod_base = OTHER; note = 2'-O-Methyl nucleotide
  modified_base 17: mod_base = OTHER; note = 2'-Fluoro nucleotide
  modified_base 18: mod_base = OTHER; note = 2'-O-Methyl nucleotide
  modified_base 19: mod_base = OTHER; note = 2'-Fluoro nucleotide
  modified_base 20..21: mod_base = OTHER; note = 2'-O-Methyl nucleotide
  misc_feature 22: note = Inverted nucleotide
  source 1..22: mol_type = other DNA
gcggtcattgtcactggtcttt

SEQ ID NO: 15 - RNA, 21 nt, synthetic construct
  modified_base 1: mod_base = OTHER; note = 2'-O-Methyl nucleotide
  modified_base 2: mod_base = OTHER; note = 2'-Fluoro nucleotide
  modified_base 3: mod_base = OTHER; note = 2'-O-Methyl nucleotide
  modified_base 4: mod_base = OTHER; note = 2'-Fluoro nucleotide
  modified_base 5: mod_base = OTHER; note = 2'-O-Methyl nucleotide
  modified_base 6: mod_base = OTHER; note = 2'-Fluoro nucleotide
  modified_base 7: mod_base = OTHER; note = 2'-O-Methyl nucleotide
  modified_base 8: mod_base = OTHER; note = 2'-Fluoro nucleotide
  modified_base 9: mod_base = OTHER; note = 2'-O-Methyl nucleotide
  modified_base 10: mod_base = OTHER; note = 2'-Fluoro nucleotide
  modified_base 11..13: mod_base = OTHER; note = 2'-O-Methyl nucleotide
  modified_base 14: mod_base = OTHER; note = 2'-Fluoro nucleotide
  modified_base 15: mod_base = OTHER; note = 2'-O-Methyl nucleotide
  modified_base 16: mod_base = OTHER; note = 2'-Fluoro nucleotide
  modified_base 17: mod_base = OTHER; note = 2'-O-Methyl nucleotide
  modified_base 18: mod_base = OTHER; note = 2'-Fluoro nucleotide
  modified_base 19..21: mod_base = OTHER; note = 2'-O-Methyl nucleotide
  misc_feature 19..21: note = Phosphorothioate linkage
  source 1..21: mol_type = other RNA
gaccagtgacaatgaccgctt

SEQ ID NO: 16 - DNA, 22 bp, synthetic construct
  misc_feature 1..21: note = RNA
  misc_feature 22: note = DNA
  misc_feature >1: note = 5' NH2-(C6H12)-linker
  modified_base 1: mod_base = OTHER; note = 2'-O-Methyl nucleotide
  modified_base 2: mod_base = OTHER; note = 2'-Fluoro nucleotide
  modified_base 3: mod_base = OTHER; note = 2'-O-Methyl nucleotide
  modified_base 4: mod_base = OTHER; note = 2'-Fluoro nucleotide
  modified_base 5: mod_base = OTHER; note = 2'-O-Methyl nucleotide
  modified_base 6: mod_base = OTHER; note = 2'-Fluoro nucleotide
  modified_base 7: mod_base = OTHER; note = 2'-O-Methyl nucleotide
  modified_base 8: mod_base = OTHER; note = 2'-Fluoro nucleotide
  modified_base 9: mod_base = OTHER; note = 2'-O-Methyl nucleotide
  modified_base 10: mod_base = OTHER; note = 2'-Fluoro nucleotide
  modified_base 11: mod_base = OTHER; note = 2'-O-Methyl nucleotide
  modified_base 12: mod_base = OTHER; note = 2'-Fluoro nucleotide
  modified_base 13: mod_base = OTHER; note = 2'-O-Methyl nucleotide
  modified_base 14: mod_base = OTHER; note = 2'-Fluoro nucleotide
  modified_base 15: mod_base = OTHER; note = 2'-O-Methyl nucleotide
  modified_base 16: mod_base = OTHER; note = 2'-Fluoro nucleotide
  modified_base 17: mod_base = OTHER; note = 2'-O-Methyl nucleotide
  modified_base 18: mod_base = OTHER; note = 2'-Fluoro nucleotide
  modified_base 19..21: mod_base = OTHER; note = 2'-O-Methyl nucleotide
  misc_feature 22: note = Inverted nucleotide
  source 1..22: mol_type = other DNA
gcggtcattgtcactggtcttt

SEQ ID NO: 17 - RNA, 21 nt, synthetic construct
  modified_base 1: mod_base = OTHER; note = 2'-Fluoro nucleotide
  modified_base 2: mod_base = OTHER; note = 2'-O-Methyl nucleotide
  modified_base 3: mod_base = OTHER; note = 2'-Fluoro nucleotide
  modified_base 4: mod_base = OTHER; note = 2'-O-Methyl nucleotide
  modified_base 5: mod_base = OTHER; note = 2'-Fluoro nucleotide
  modified_base 6: mod_base = OTHER; note = 2'-O-Methyl nucleotide
  modified_base 7: mod_base = OTHER; note = 2'-Fluoro nucleotide
  modified_base 8: mod_base = OTHER; note = 2'-O-Methyl nucleotide
  modified_base 9: mod_base = OTHER; note = 2'-Fluoro nucleotide
  modified_base 10: mod_base = OTHER; note = 2'-O-Methyl nucleotide
  modified_base 11: mod_base = OTHER; note = 2'-Fluoro nucleotide
  modified_base 12: mod_base = OTHER; note = 2'-O-Methyl nucleotide
  modified_base 13: mod_base = OTHER; note = 2'-Fluoro nucleotide
  modified_base 14: mod_base = OTHER; note = 2'-O-Methyl nucleotide
  modified_base 15: mod_base = OTHER; note = 2'-Fluoro nucleotide
  modified_base 16: mod_base = OTHER; note = 2'-O-Methyl nucleotide
  modified_base 17: mod_base = OTHER; note = 2'-Fluoro nucleotide
  modified_base 18: mod_base = OTHER; note = 2'-O-Methyl nucleotide
  modified_base 19: mod_base = OTHER; note = 2'-Fluoro nucleotide
  misc_feature 19..21: note = Phosphorothioate linkage
  modified_base 20..21: mod_base = OTHER; note = 2'-O-Methyl nucleotide
  source 1..21: mol_type = other RNA
gaccagtgacaatgaccgctt

SEQ ID NO: 18 - DNA, 22 bp, synthetic construct
  misc_feature 22: note = DNA
  misc_feature 1..21: note = RNA
  modified_base 1: mod_base = OTHER; note = 2'-Fluoro nucleotide
  modified_base 2: mod_base = OTHER; note = 2'-O-Methyl nucleotide
  modified_base 3: mod_base = OTHER; note = 2'-Fluoro nucleotide
  modified_base 4: mod_base = OTHER; note = 2'-O-Methyl nucleotide
  modified_base 5: mod_base = OTHER; note = 2'-Fluoro nucleotide
  modified_base 6: mod_base = OTHER; note = 2'-O-Methyl nucleotide
  modified_base 7..9: mod_base = OTHER; note = 2'-Fluoro nucleotide
  modified_base 10: mod_base = OTHER; note = 2'-O-Methyl nucleotide
  modified_base 11: mod_base = OTHER; note = 2'-Fluoro nucleotide
  modified_base 12: mod_base = OTHER; note = 2'-O-Methyl nucleotide
  modified_base 13: mod_base = OTHER; note = 2'-Fluoro nucleotide
  modified_base 14: mod_base = OTHER; note = 2'-O-Methyl nucleotide
  modified_base 15: mod_base = OTHER; note = 2'-Fluoro nucleotide
  modified_base 16: mod_base = OTHER; note = 2'-O-Methyl nucleotide
  modified_base 17: mod_base = OTHER; note = 2'-Fluoro nucleotide
  modified_base 18: mod_base = OTHER; note = 2'-O-Methyl nucleotide
  modified_base 19: mod_base = OTHER; note = 2'-Fluoro nucleotide
  modified_base 20..21: mod_base = OTHER; note = 2'-O-Methyl nucleotide
  misc_feature 22: note = Inverted nucleotide
  source 1..22: mol_type = other DNA
gcggtcattgtcactggtcttt

SEQ ID NO: 19 - RNA, 21 nt, synthetic construct
  modified_base 1: mod_base = OTHER; note = 2'-O-Methyl nucleotide
  modified_base 2: mod_base = OTHER; note = 2'-Fluoro nucleotide
  modified_base 3: mod_base = OTHER; note = 2'-O-Methyl nucleotide
  modified_base 4: mod_base = OTHER; note = 2'-Fluoro nucleotide
  modified_base 5: mod_base = OTHER; note = 2'-O-Methyl nucleotide
  modified_base 6: mod_base = OTHER; note = 2'-Fluoro nucleotide
  modified_base 7: mod_base = OTHER; note = 2'-O-Methyl nucleotide
  modified_base 8: mod_base = OTHER; note = 2'-Fluoro nucleotide
  modified_base 9: mod_base = OTHER; note = 2'-O-Methyl nucleotide
  modified_base 10: mod_base = OTHER; note = 2'-Fluoro nucleotide
  modified_base 11..13: mod_base = OTHER; note = 2'-O-Methyl nucleotide
  modified_base 14: mod_base = OTHER; note = 2'-Fluoro nucleotide
  modified_base 15: mod_base = OTHER; note = 2'-O-Methyl nucleotide
  modified_base 16: mod_base = OTHER; note = 2'-Fluoro nucleotide
  modified_base 17: mod_base = OTHER; note = 2'-O-Methyl nucleotide
  modified_base 18: mod_base = OTHER; note = 2'-Fluoro nucleotide
  modified_base 19..21: mod_base = OTHER; note = 2'-O-Methyl nucleotide
  misc_feature 19..21: note = Phosphorothioate linkage
  source 1..21: mol_type = other RNA
gaccagtgacaatgaccgctt

SEQ ID NO: 20 - DNA, 23 bp, synthetic construct
  misc_feature 1: note = DNA
  misc_feature 2..22: note = RNA
  misc_feature 1: note = Inverted nucleotide
  modified_base 2: mod_base = OTHER; note = 2'-Fluoro nucleotide
  misc_feature 1^2: note = Phosphorothioate linkage
  modified_base 3: mod_base = OTHER; note = 2'-O-Methyl nucleotide
  modified_base 4: mod_base = OTHER; note = 2'-Fluoro nucleotide
  modified_base 5: mod_base = OTHER; note = 2'-O-Methyl nucleotide
  modified_base 6: mod_base = OTHER; note = 2'-Fluoro nucleotide
  modified_base 7: mod_base = OTHER; note = 2'-O-Methyl nucleotide
  modified_base 8..10: mod_base = OTHER; note = 2'-Fluoro nucleotide
  modified_base 11: mod_base = OTHER; note = 2'-O-Methyl nucleotide
  modified_base 12: mod_base = OTHER; note = 2'-Fluoro nucleotide
  modified_base 13: mod_base = OTHER; note = 2'-O-Methyl nucleotide
  modified_base 14: mod_base = OTHER; note = 2'-Fluoro nucleotide
  modified_base 15: mod_base = OTHER; note = 2'-O-Methyl nucleotide
  modified_base 16: mod_base = OTHER; note = 2'-Fluoro nucleotide
  modified_base 17: mod_base = OTHER; note = 2'-O-Methyl nucleotide
  modified_base 18: mod_base = OTHER; note = 2'-Fluoro nucleotide
  modified_base 19: mod_base = OTHER; note = 2'-O-Methyl nucleotide
  modified_base 20: mod_base = OTHER; note = 2'-Fluoro nucleotide
  modified_base 21..22: mod_base = OTHER; note = 2'-O-Methyl nucleotide
  misc_feature 23: note = Inverted nucleotide
  source 1..23: mol_type = other DNA
  misc_feature 23: note = DNA
tgcggtcattgtcactggtcttt

SEQ ID NO: 21 - RNA, 21 nt, synthetic construct
  modified_base 1: mod_base = OTHER; note = 2'-O-Methyl nucleotide
  modified_base 2: mod_base = OTHER; note = 2'-Fluoro nucleotide
  modified_base 3: mod_base = OTHER; note = 2'-O-Methyl nucleotide
  modified_base 4: mod_base = OTHER; note = 2'-Fluoro nucleotide
  modified_base 5: mod_base = OTHER; note = 2'-O-Methyl nucleotide
  modified_base 6: mod_base = OTHER; note = 2'-Fluoro nucleotide
  modified_base 7: mod_base = OTHER; note = 2'-O-Methyl nucleotide
  modified_base 8: mod_base = OTHER; note = 2'-Fluoro nucleotide
  modified_base 9: mod_base = OTHER; note = 2'-O-Methyl nucleotide
  modified_base 10: mod_base = OTHER; note = 2'-Fluoro nucleotide
  modified_base 11..13: mod_base = OTHER; note = 2'-O-Methyl nucleotide
  modified_base 14: mod_base = OTHER; note = 2'-Fluoro nucleotide
  modified_base 15: mod_base = OTHER; note = 2'-O-Methyl nucleotide
  modified_base 16: mod_base = OTHER; note = 2'-Fluoro nucleotide
  modified_base 17: mod_base = OTHER; note = 2'-O-Methyl nucleotide
  modified_base 18: mod_base = OTHER; note = 2'-Fluoro nucleotide
  modified_base 19..21: mod_base = OTHER; note = 2'-O-Methyl nucleotide
  misc_feature 19..21: note = Phosphorothioate linkage
  source 1..21: mol_type = other RNA
gaccagtgacaatgaccgctt

SEQ ID NO: 22 - RNA, 21 nt, synthetic construct
  misc_feature 1: note = Inverted abasic capped nucleotide
  modified_base 1..2: mod_base = OTHER; note = 2'-O-Methyl nucleotide
  modified_base 4: mod_base = OTHER; note = 2'-O-Methyl nucleotide
  modified_base 10: mod_base = OTHER; note = 2'-O-Methyl nucleotide
  modified_base 14: mod_base = OTHER; note = 2'-O-Methyl nucleotide
  modified_base 20..21: mod_base = OTHER; note = 2'-O-Methyl nucleotide
  source 1..21: mol_type = other RNA
gcggtcattgtcactggtctt

SEQ ID NO: 23 - RNA, 21 nt, synthetic construct
  modified_base 20..21: mod_base = OTHER; note = 2'-O-Methyl nucleotide
  source 1..21: mol_type = other RNA
gaccagtgacaatgaccgctt